European Patent Specification EP 3 430 173 B1, published September 18, 2024. Title: A method for the production of a dairy food product and a method for gene transfer by conjugation. Applicant: Stichting Top Institute Food and Nutrition. The sequence listing filed with the application follows.

SEQUENCE LISTING (6 sequences)

SEQ ID NO: 1 - DNA, 7714 bp, Lactococcus lactis
atgaagaaaaagtgggcgacttggctcagccttttggtactatgtttgagtatagtagcaaatattagccaaggatacacagtattagcagattcatctaattcactaacctcaggggatccaaccacagcagatccatttaattatataaaaaatggtgatgtggcttatccaaaacaaggcacatcaacttatcaaaatggcaaaacagatgaagatatcgtaaactatgatttttcacaatcaagcagtgaaggccagtctagcataaaaaatattttcggaagtggggcacttacttttgataacggctatcattattatcaaaatgatgggtatgttaagaagatagttatgcctactaatgatcccacccaatttaaagtccgtttagatatgataggtgaggagttaaaaacaaccaaacctgttgacatcgccatggtattagataattcaacgtcaatgaattatgatatgggagcagggaagacaagatggcagactttgaaagactctgttaaaaattttgctaaccaattaattggtccatcttcaaataataatgataatgtaagaataggcttttcaagttttggttctgagcggcaaaggattagtatttggccaggttattctgatataccatttacaaaaattggtaaattttcatcaaactcatcttttacctctaactatactcagttattgaattcaagtatttatactcctacagcagcaccaaggctttctggtaccccgacatttttaggtgtagatgcaggatataagatgttgtcagatgctacatatggtgcacgttctgattcagtaaaagtattgattgttctaacagatggagaaccgacattttggaattcaggatcctacactagcttaagtaatgtgggatcaacgactaattatgattatttttcaactccgtattattctggtaatggagtgaaatctgaatctaattatacgagtacaataaattttgtcaatcaaagagccaatgcgaatccaggagtatcaaagtattcgattggtatttctacagttaataacagtggcataaaatcagtcttaaaggcgctaggaccagatggtacttttgaagcgtcaaatcaacaagatctagtggatgctttagacaaaattaggacgtcgattagtaagtctattcaaaaaggctcattgattgaccctatgagtcagtatgtcacgttaaatacgaacagcatacagacatatgatttgaaagttgatagtaatagtatatcagcgacaggctcaaatcgtagtgttaaaactgataataaccaaatctctattgataatttaagtattggtaaaaatgaaggagtacgtgtagagtatacagtctccttaaaacaacaatattgggatggacagtttcatccagctaacggcacaacttatttacaaaataataagttatcaccagctcaatatcttcattttgcagttccatccattaagtatgatacttttaatctaccagttcaaaaaatttgggatgatcaaaataaccagtatcaaacgagacaagatattatcttacaactacaatcttttgtgaacaatacatggcaaaatgtatctgataagacatttgccattaaggcaagtgcgacagatgatcaactcaaaggtgttatttctggtattccatccaaggatggtgcaaatcaaccaattaaatatcgacttgttgagttgtttggaaatactgagcaagcagttaatggttatgctacaccaagttattcaacgccaagggaaataacatatacagatatagttaatggtaatgtgtctaaagacaagccgttagctgtaacaaatacattattaaaaacagctattagttttacaaaagttggtaatgataatcagactcctttagcaggagctgagtttaccctttatgcctctgatggaaaaacacaaattggatcgccagtcacgtctgataaaaatggcctagttaaattcgatcaacaagtaccaattgggaaatacttaatcaaagaaactaaaacaccacttggttatgtcaaagcttctgatattaatatttcggtaactgctcaaaatggacaacttgtcatttcaggtttgccaactggcagtaaggttaaaaatatattagatgatttcaaattaattatcactaaaaaagataataatggcaatgctgtatctggtgttaaatttaaacttgttggttcaaataattataataaggaacaagaatctgatgctagtaatggaaatgtatttacttttcaagggttaaaaccaggcaagtatgcattaactgagactaaaacaccagaaaaatatgttggtctaaaacaagatgtgatcattttgattggggacgatggtaaagtcactattgatggacagccgctacctgatcaaccaattaccacaactggtaatatcattaagcttgatgtgacgaatacgataaaaggtattctccctagtacaggtggctctggtcggacaggctattttatagcgagtcttatctttatgggattagttgcgattatcggtggtatcttctactatcgtaatagacgtctacgtcatcataaacttcttaaaggtccacataacaaaagtcatctgttactgttgctgttaatcacgtctctgggaataacctttacaaatgctcagaaaatagcagcagatgaacaaccgattacctttatcttacataaacgtgtctttaaagatagtggagacttaaaaacaattaaagataatgggttagtgattacacctaatgatcccaattcaggtgtgattgattcggataaaacatatgggttgaatggtgtcactttcgatgtttatgatgtcactagttatgtgtcaaatgctttaaaaagtacatctaaagaggcgcttatgaaacacgtcacaaatactgataaggctagcctattggccgaaataaagccatatcagccaacaagtcaggaagttgtgacggtttcaagcgatggagatgatggtgttgcacgatttagtgttcaacctacttctcaaaacagtgcttatctgatactggagaagcagatctctgacaaagatgctggtaaagtcaagatgacggcaacaccgatgttggttatattaccagtagcgaatcctgttgataaaacatcatttttgacaacgataaatctgtatcctaaaaatacagcagtcaaaacaccagttatcccaccagtaaacccggtaaatccgaaaccacctcatttcccttttttacctgatacaggtgaagttaagtcggtaatggttgttttgggtggcattgtcgtaatcatagcagttagcttttggtataaccgacgtaagccaaagccgtcataaactaaagtctttgtcaattattgtcaagcttatatagaaaattttggagaaaaatatgaaaacaaacaaattcttacaagtgattttagcaacaattttgttgttaacaaccgcttttgtgtcaaatcagcatattatttagtaataataaggaaaaattaagatgatcttttatagattgattttgaaaggagatagggacacaccttaaaacgaagcacagtgtaaaaatcactcactcaaaaatggagaataaaatgaaaaaagaaaaattattaaaattagtaatgacgttattgctagcgttgatagctattgttgccccaatttcatctgcttttgcggatgacacaattgatgactctacaaaggttaatgtgaccttaaataaactgatttggaatgataatgcaccaactgatttccaaaatacaggtgcaaaaatgaactttgacggttcagctacaccattaaatggatctgaatttacgctttatgatgttacaagtcaatattataactatattgctaataagagccaacaagcagccattagccaaattcaagcagacgcaagtcaagttgctccaaattatgcaaaaaacattaaatcagttaccactgctgggcaaggacaggctttattcaatgatttgtcagtaaagaataaatcaggacaatataacgtttatcttttccttgaaactaaaacccctgacaatattacagttacaaaattgtcagctcctattgtgttggcaatgccgatttacactttagataaacaacaacaacctactgacacactaaatcaagacattcaactttatcctaaaaacgttacatctaaagatacaaaagaatttacaaatgttggatcatttagtaaggtaactgttggagatcagtcttttgctaatgtgacaacaggcgatgttttaaactatactttgaccgttaacattcctgctaatattggtgatgcaaatgctgttaataaatattcgatttttgataaaccatctgatggacttgcactcgttaacaatacagttactgtgggaagtttgactgcgggaaatggaacttcagaggattatgatattgcttatgtaaatggtggattcacggttaatttacatctgaacagtgataatgttaaagcattggctggtaaaaaaatacaattaacttataatatgaaattgacggcagatgtgaatccggataatttacaaagtaacaaagcgagtgtccaaattaataattcgcctgaacaacaaatcacccctccaactcctgtaggtactggtggttacaaatttatcaaaaaggatgctcaaactggaaaaaacttatctggggcagagtttgtcgtggctaatagtgataaatcaaaatttgcaaaatttagtggtcaaaactcaaaaagtgaatatgtatttgattcatgggtctcaaaagatcaagcaacaaaaattgtttccggaaatgatggatcattcaatgtaatcggacttacaaatgggaattacgtacttaatgaaactaaagcaccttcagctaactatgttctcttaaaagatggtacaattacatttacagttgtacatggtaaatatgtcacatcaaacttagatgttaagaatacacctaaagggctattgccatcaactggtggtgctggtatctacgccttcatcattattggtgcagcaatgatgattggtgcatatatttggtttaaaaaatcaagacaacaagcagaagtttaagtctttagactaacaggttttttcctgaagttaaaggttaacgttaacaaggctggggaactttcccagccttgttgtgtttcggaaaggaaggtgtatcagcattgaaaaaacaatacccgcagcaagataacttaaaaaacgaaagaatcaatttatggcttaaggttttgatggcgcttttgttctttgcaggtgcaatggtattttcctacccttttgttgtcgatacaatcaataatttttatgatcaacgtgtgattgataactatcaaatccaatatcaaacagcacataaagcgcaacaaaaaaaacagttggcccagatgaaagcagaaaatgaatccttgctcaaacaagagcatacgacaaacattcctggcatgggcttagttgaagatccgtttgaaagtgcactaaaaaataatgtgaaaccaagcaaagcttatttgcaatctcatatgataggtgccatttttattccttctatccatgttagtttacctatttttaatgaaactaacgacgagttattagaaaaaggcgctacagtattacaggggacttcttatccgataggtggtatcagtacacattcagttttgactgggcacagtggtctaccagataaaaaactctttacggatttggataaactgaaaaaaggtgacttattttatattgaagtattgggtgagaaattagcttatcgtgcagttaactttaaaacggtattaccaacacaactagagagtttaaagatagtggatggcaaagatttagtcactttagtgacttgtaccccttatatggttaatacgcatcgtttattagtcacgggagaacgtgttccttttgtcgaacaaaagatgaccaagcaaatcaaaaaagcacaagcctatcatcagaatagactactcgcttttgcagtcggtattccgattttctgtttattatttgcatattttatatggcgcaagtttgtctattatctgtgtatcaaacatcgctatgattttgtattctacgctgtagctaatggacaaggaatagctaatttagccttttatctgatagagaaaaaagggaaaataccagtattaagagacggtgaacggcttaaagcaatcagtgataaagatgggcgtgtcctgtttgaagatatcccaggtggccgctatgttgcttatcctgatgagcaaaccgcttttccaaaagtatctggatttgtgcgactgttacaggatcaacactttacacttaagtctcatggtgcacgcgtaaaaagaaccggtaagcaacaccatcgtgactatatcattgataggggacatcatgcgaaataaaaacaagccacaaggaaaggctaaaaaaagcataggcaagcgttttttgattaatttgatggtttatagtttatttttgattggtatattgatcatgctatatccgttttatatcagtgccttaaatgactacttagataatgttcgcgtgtcgctttataaggatagtttacaaaaagctcacgacacacaagaaaagcagttgaaagcagctaatgaaaaattagctaaacaaggcttgacaccctctaaagatccttttaaagatgacaaagcaagtggtgtttctgaagattattataaaaaacatctactaggcaccattgatattcctaagatcaacattaaaatcccactatttgatacgactaatagtgaactgttagaaattggtgcaacaaccttaaatgggacctcatacccattaggaggtcaaaatacacacgctgtgattgcggctcatcgagggctaccagaccgtgcactttttactgatttaccaaaactaaaagaaggggatatctttgttttagaagtattgggtcataagttagcctatgaggtgaagacgattgttgtggtgaaaccagaagaaacacaggtcttaaagatagagccagggcaagacttggtgacgttattgacttgtacaccttatatgatcaactctcatcgcttactagtaactggcagtcgtgtcccttatacgcccaaagttgaaaagatgttagcgcaaaatgaccataatcgcaaactgatccaacttgctttgctagtcttatttaccttactagtttgcttaatgctctggatactttatcgtattatccaccaatacctgctcactaagcaaaatatgtcgattattttacagattatcacctcagatcaatcgccttacgcacaacctttacatctttatgatcgaacgggtaaaagagcattgaagcgtcaaggtgaggcggtgatattaataccagatgcgacgggtacttatcagattgatcacttagcaaaagggatgtattgtttaaaaaccaaagatgatgcgctatgtgtgttgatcggacaaactaagataaaagcgatgacttatcaacttaaagtaatgaaaagatctaaattatcctttaaacaactctcaaagcaagtaattcaaattactta

SEQ ID NO: 2 - DNA, 383 bp, Lactococcus lactis
tttccatgaataaaaggattttttatttttctttttccaaatttgatagtagatttaaaactttgcaacagaaccgtaattgattagcaaaaatatttttttcaaataagatagataaatcagtgtaaaatcgacaaataaggtcttgcattttctatagaattgatatatagttaattagatcggcagttactgatgaaacaggctataccttgaaatgtactcgatttatcgagtattatgatataaatctagatgatataaattaaaaagttgagcgtaataattgttttgagtttccaaccgaattaagctgttttcagatctttgatcggtgtcaagatttgcttacatatatattttaagagaaagggggacgatat

SEQ ID NO: 3 - DNA, 24 bp, Artificial Sequence
  PCR primer
ggaccagatggtacttttgaagcg

SEQ ID NO: 4 - DNA, 26 bp, Artificial Sequence
  PCR primer
ggtaaagtcactattgatggacagcc

SEQ ID NO: 5 - DNA, 36 bp, Artificial Sequence
  PCR primer
ccgctgcagtttgcaacagaaccgtaattgattagc

SEQ ID NO: 6 - DNA, 50 bp, Artificial Sequence
  PCR primer
cggctcgagttaagtaatttgaattacttgctttgagagttgtttaaagg